European Patent Application EP 4 212 621 A1, published July 19, 2023. Title: Glycoside hydrolase for synthesis of xylose oligosaccharides. Applicant: Max-Planck-Gesellschaft zur Förderung der Wissenschaften e.V. The sequence listing filed with the application follows.

SEQUENCE LISTING (11 sequences)

SEQ ID NO: 1 - protein, 323 aa, Rhamnusium bicolor
  Rbic4 (1)..(323)
MNSLLLISLAILGCIINIATSLDAALETVSKHGKLSVNGIQLTDSHGQAVQLKGMSLFWSVWMPYYWNRPTVDSIHSACHSNIVRAAMAVENDGYLTHPDVEMERVETIIEAAIADDIYVIVDWHDSESEKYLSESKDFFDKISKKYGRYPNIIYETYNEPIGQSWSAVIKPYHQSVINTIRANDPDNVILLGTPHYNQEYDSVINDPITGQRNIMYTLHFYSNEGGNDQLRDRADKAMSAGLPIFVTEYGTSMGSGNGTVDAAATQVWYDWLDGNGISYVNWALSDKDESASSQIAGTPPEQACRDNYLTESGRIVVAQNRK

SEQ ID NO: 2 - protein, 323 aa, Rhamnusium bicolor
  Rbic5 (1)..(323)
MNSSLLISLAILSCIINIATSLDAAQETVSKHGKLSVNGIRLTDSHGQPVQLKGMSLFWSVWMPYYWNRATVDSIHKACHSNIVRAAMAVENDGYLTHPDVEMERVETIIEAAIANDIYVIVDWHDSDSEKHLAESKDFFDKISKKYGRYPNIIYETYNEPISQSWSAVIKPYHQSIISTIRSNDQDNVIIVGVPHFDQEYDQAINDPITGQRNIMYTLHFYSNEGGNDQLRDRADKAMSAGLPIFVTEYGTSMGSGNGTVNAAATQVWYDWLDRNGLSYVNWALSDKDESASSQKAGTPPEQACQDNYLTESGRIVVAQNKK

SEQ ID NO: 3 - DNA, 972 bp, Rhamnusium bicolor
atgaattctttacttctaatttcgttggccatattgggctgcataatcaacatcgctacttcgcttgatgctgcactagagactgtaagtaaacatggtaaactttccgttaatggtatccagttgacggattctcatggtcaggcggtgcaactaaaaggaatgtcattattttggagtgtttggatgccatactactggaatagaccgactgtagactcaattcatagtgcatgccattccaatatagttcgagcagcgatggcggtcgaaaatgatggatatttgacacatccagacgtggaaatggagagagtggagacaattattgaagcggcaatcgcggacgatatatacgtgattgtagattggcacgattcagaatcagaaaaatatttgtcagagtcaaaggatttctttgataaaatctcgaagaaatatggtaggtacccgaacattatttacgagacttacaacgaacccattggacaatcatggagtgccgttataaagccctaccatcaatctgtaatcaacaccattcgagccaacgatccagataatgtgatattattaggcacgcctcactacaaccaagagtacgattcggtgattaacgatccgattactggccaaagaaacattatgtacacactacatttctactctaacgaaggcggaaacgatcagctacgagacagggcagacaaagcaatgagtgcaggacttccaattttcgtaacggaatacggtacttctatgggatccggaaacggtaccgtagacgcggctgcaactcaagtatggtatgactggctggacggaaatggaatatcttatgtcaactgggccctctccgataaggatgagagcgcatcttcacagatagcaggaacacccccagaacaagcttgccgggataattatttgaccgaatccggaaggatagtcgtagcgcaaaacagaaaatag

SEQ ID NO: 4 - DNA, 972 bp, Rhamnusium bicolor
atgaattcctcacttctaatttcgttggccatattgagctgcataattaacatcgctacttcacttgatgctgcacaggagaccgtaagtaaacatggtaaactttctgttaatggtatccggttgacggattcgcatggtcaaccggtgcaactaaaaggaatgtcactattttggagtgtttggatgccatactactggaatagagcgaccgtagactcaattcataaggcatgccattccaatatagttcgagcagcgatggcagtcgaaaatgatggatatttgacacatccagacgtggaaatggagagggtggagacaattattgaagcggcaatcgcgaatgatatatatgtgattgtagattggcacgattctgactcagaaaaacatttggcagagtcaaaagatttctttgataaaatctcgaagaaatatggtaggtacccgaacattatttacgagacttacaacgaacccatttcacaatcatggagtgccgttataaagccctaccatcagtcaataatcagcaccattcgatccaacgatcaagataatgtgatcatagtaggtgtgcctcactttgatcaagagtacgatcaggcgattaacgatccaattaccggccaaagaaacattatgtacacactacatttctactctaacgaaggcggaaacgatcagctacgagacagggcagacaaagcaatgagtgcaggacttccaattttcgtaacggaatacggtacttctatgggatccggaaacggtacagtaaacgcggctgcaactcaagtatggtatgactggctggacagaaatggattatcttatgtcaactgggccctctccgataaagatgagagcgcatcttcacagaaagcaggaacacccccagaacaagcttgccaggataattatttgaccgaatccggaaggatagtcgtagcgcagaacaaaaaatag

SEQ ID NO: 5 - DNA, 972 bp, Artificial Sequence
  Rbic5_synthetic-construct
atgaactccagcctgctgatctcactggctatcctgtcctgcatcatcaacatcgccacctcactggacgctgcccaggagactgtgtcaaagcacggaaagctgtccgtcaacggtatcaggctcactgactcccacggccagcctgtgcagctgaagggaatgagcctgttctggtctgtctggatgccctactactggaacagggctactgtggacagcatccacaaggcctgccactctaacatcgtgagagctgctatggctgtcgaaaacgacggttacctgacccaccctgacgtggagatggaacgcgtcgagactatcatcgaagctgccatcgctaacgacatctacgtgatcgtggactggcacgactccgacagcgagaagcacctggccgaatcaaaggacttcttcgacaagatctccaagaagtacggccgttacccaaacatcatctacgagacctacaacgaacctatctctcagtcatggtccgctgtcatcaagccataccaccagagcatcatctctactatccgctccaacgaccaggacaacgtgatcatcgtgggcgtcccccacttcgaccaggagtacgaccaggccatcaacgacccaatcaccggacagcgtaacatcatgtacactctgcacttctacagcaacgagggtggcaacgaccagctgagggacagggctgacaaggctatgtctgccggtctgcctatcttcgtcaccgaatacggcactagcatgggttccggtaacggcaccgtgaacgctgccgctactcaggtctggtacgactggctggacaggaacggtctgagctacgtgaactgggctctgagcgacaaggacgaatctgcttcttcacagaaggctggaacccctcccgagcaggcttgccaggacaactacctgactgaatccggtagaatcgtggtcgcccagaacaagaagtaa

SEQ ID NO: 6 - protein, 322 aa, Rhamnusium bicolor
  Rbic9 (1)..(322)
MNSSLLTSLVILCCIINIATSLDAALETVSKHGRLSVSGTQLMDSHGQPVQLKGMSLFWSVWMPYYWNRATVDSIHSACHSNIVRAAMAIEYEGYLDHPDVEMQRMETIIEAAIANDIYVIVDWHDWNGEKHLSQAKDFFDKISKKYGSYPNILYETYNEPIDISWSAIVKPYHLSVISTIRSNDPDNVILLGVPHYDQELDQAADDPITGQNNIMYTLHFYANENKQWLRDRAQNVIRQGLPIFVSEYGTCDGSGNGSIDAAETQLWYNWLDQNHMSYVNWALSDKDESASSQIAGTPPEQACQDRYLTESGRIVVAQNKK

SEQ ID NO: 7 - DNA, 969 bp, Rhamnusium bicolor
  Rbic9 (1)..(969)
atgaattcctcacttttaacctcgttagtcatattgtgctgcataatcaacatcgccacttcgcttgatgctgcactggagaccgtaagtaaacatggtagactttccgttagtggtacccagttgatggattcgcatggtcagccggtgcaacttaaaggaatgtcactattttggagtgtttggatgccatactattggaatagagcgaccgtagactcaattcacagtgcatgtcattccaatatagttcgagcagcgatggcgattgaatatgagggatatttggatcatccagatgtggaaatgcagaggatggagactattattgaagcagccattgcgaatgatatatatgtgatcgttgattggcacgactggaacggagaaaaacatttgtcacaagcgaaggatttcttcgataaaatctcaaagaaatatggtagctacccaaacattctttacgagacctacaacgaacccattgatatatcatggagtgccattgtaaagccctaccatctgtcagtaatcagcactattcgatccaacgatccagataatgtaatcttactaggcgtgccccactacgatcaagagttggatcaggcggctgacgatccgattaccggccaaaataacattatgtacacactacatttctacgctaacgaaaacaaacagtggcttcgagacagggcacaaaacgtaattcgtcaaggacttccaattttcgtatcggaatatggtacttgtgatggatccggaaacggttccattgacgcggctgaaactcaattatggtataactggctggaccaaaatcatatgtcttatgtcaactgggctctttccgataaggatgagagcgcatcttcacagatagcaggaacacccccagaacaagcttgccaggatcgttatttgaccgaatccggaaggatagtcgtagcgcagaacaaaaaatag

SEQ ID NO: 8 - protein, 320 aa, Apriona japonica
  Ajap1 (1)..(320)
MKTFFILSCLVVLINNSLSKDAAQETVSKHGKLSVQGTQLVNQNGEAVQLKGMSMFWSVWMPKYWNEATVQSIHNACHSNIVRAAMAVEYGGYLTDPTTEMQRVETVIEAAIKNDIYVIADWHDWHAEEHLEQAKGFFEQISKKYGGYPNLIYETYNEPLDIAWSSVVKPYHEEIIKVIRANDPDNVILLGSPHYDQELDQVLADPITGQTNIMYTLHFYSVDTKQWLRDRVQNVMNNGIPIFVSEYGTCAGTGNGTVLADETQLWWDWLDQNQMSYVNWALSDKDEAASVLIADTTPENACQDAYLTESGKLVIPQNKK

SEQ ID NO: 9 - DNA, 963 bp, Apriona japonica
  Ajap1 (1)..(963)
atgaagacgttttttattttatcgtgcttggtcgtactgatcaacaacagtttgtcgaaagatgctgcccaggaaactgtgagcaagcacggcaagttatccgtccaaggtactcaattggttaatcaaaatggcgaagccgtgcaattgaaaggtatgtccatgttctggagcgtatggatgccaaaatactggaatgaagctaccgtccaatcaattcacaacgcttgtcattccaacattgtccgcgctgctatggctgtcgaatacggtggatacttgactgacccaactactgaaatgcaaagggtggagacagttatcgaagcagccattaagaacgacatttacgtaatcgccgactggcatgattggcacgccgaggaacatttggaacaggccaaaggtttctttgaacaaatctctaagaaatacggaggttacccaaatctcatctacgagacatacaacgaacccctcgatatcgcatggtccagcgttgtgaagccctaccacgaggaaatcattaaagtcatccgtgctaacgatcccgataatgtcatcttgttgggttcgccacactatgatcaggaattggaccaagtactagctgatccaatcactggtcaaaccaacattatgtacactcttcatttctactctgttgataccaagcaatggttaagggatagagtccaaaacgtaatgaacaacggaatcccgatcttcgtatctgaatatggcacatgcgcaggaaccggaaacggaacagttttggctgatgagacccaactttggtgggattggttagaccagaaccagatgtcttatgtcaactgggccctttctgacaaggatgaagccgcatctgtattaattgcagatactactccagaaaacgcttgccaagatgcatacctgactgaatccggaaaactcgttattcctcaaaataagaaataa

SEQ ID NO: 10 - protein, 322 aa, Anoplophora glabripennis
  Agla1 (1)..(322)
MKSLLLFCLVVLGTLINQSSSKDAAQETVSKHGKLSVKGTQLVNQNGEALQLKGMSLFWSVWMPKYWTKPTIDSVHNYCHSNIVRAAMAVEYDGYLTDPTTQMQMVETVIEAAIQNDIYVIADWHDWHAEQHLEQAKGFFEQISKKYGGYPNLIYETYNEPLDIAWSSVVKPYHEEIIKVIRANDPDNIILLGSPHYDQELDQVLADPIQGQTNIMYTLHFYPVDTKQWLRDRIQNVMNNGLPIFVSEYGTCAGTGNGTVEAAETQLWWDWLDQNQMSYVNWALSDKDESASALIANTPAEQACQDQYLTESGKLVIPQNKK

SEQ ID NO: 11 - DNA, 969 bp, Anoplophora glabripennis
  Agla1 (1)..(969)
atgaagtcacttctgctgttttgtttagttgtactgggcaccttgatcaaccagagctcatcgaaggatgccgctcaggaaaccgtaagcaagcacggtaaactgtccgtaaagggtacccaattggtcaaccaaaatggtgaagccctacagttgaaaggtatgtccctattctggagcgtatggatgcctaaatactggactaaacccaccatcgactcggtccacaactactgccactcaaatatcgtccgtgctgctatggccgttgagtatgatggctacttgaccgacccaactacccaaatgcaaatggtggaaaccgttatcgaggcagctatccagaatgacatctacgtaattgctgattggcacgattggcacgcggaacaacatttggaacaagccaaaggattctttgagcagatctcgaagaaatacggcggttacccaaatttgatctatgagacctacaacgaacccctcgacatcgcatggtcaagtgtcgtgaaaccctaccacgaagagatcatcaaagttattcgtgccaacgatcccgacaacataatcctgctgggttccccacattacgatcaagaattggaccaagtattagccgatcccattcagggtcagaccaacattatgtacaccctccacttctaccccgtcgataccaaacaatggttgagagacagaatccaaaacgtgatgaacaatggactccctatcttcgtatctgaatacggcacttgcgccggaactggaaatggaaccgtagaagcggccgaaactcaactttggtgggactggctggaccagaaccaaatgtcttacgtcaactgggctctttccgacaaggacgaatctgcttccgcattgatcgcgaatactcctgctgaacaggcctgccaagaccaatacctgactgaatctggaaaactggtcattcctcagaacaagaaataa